European Patent Application EP 4 461 303 A2, published November 13, 2024. Title: Methods and Compositions for Treating Inflammatory Conditions. Applicant: The Scripps Research Institute. The sequence listing filed with the application follows.

SEQUENCE LISTING (61 sequences)

SEQ ID NO: 1 - protein, 374 aa, Homo sapiens
MKALIFAAAGLLLLLPTFCQSGMENDTNNLAKPTLPIKTFRGAPPNSFEEFPFSALEGWTGATITVKIKCPEESASHLHVKNATMGYLTSSLSTKLIPAIYLLVFVVGVPANAVTLWMLFFRTRSICTTVFYTNLAIADFLFCVTLPFKIAYHLNGNNWVFGEVLCRATTVIFYGNMYCSILLLACISINRYLAIVHPFTYRGLPKHTYALVTCGLVWATVFLYMLPFFILKQEYYLVQPDITTCHDVHNTCESSSPFQLYYFISLAFFGFLIPFVLIIYCYAAIIRTLNAYDHRWLWYVKASLLILVIFTICFAPSNIILIIHHANYYYNNTDGLYFIYLIALCLGSLNSCLDPFLYFLMSKTRNHSTAYLTK

SEQ ID NO: 2 - protein, 333 aa, Homo sapiens
GAPPNSFEEFPFSALEGWTGATITVKIKCPEESASHLHVKNATMGYLTSSLSTKLIPAIYLLVFVVGVPANAVTLWMLFFRTRSICTTVFYTNLAIADFLFCVTLPFKIAYHLNGNNWVFGEVLCRATTVIFYGNMYCSILLLACISINRYLAIVHPFTYRGLPKHTYALVTCGLVWATVFLYMLPFFILKQEYYLVQPDITTCHDVHNTCESSSPFQLYYFISLAFFGFLIPFVLIIYCYAAIIRTLNAYDHRWLWYVKASLLILVIFTICFAPSNIILIIHHANYYYNNTDGLYFIYLIALCLGSLNSCLDPFLYFLMSKTRNHSTAYLTK

SEQ ID NO: 3 - protein, 53 aa, Homo sapiens
GAPPNSFEEFPFSALEGWTGATITVKIKCPEESASHLHVKNATMGYLTSSLST

SEQ ID NO: 4 - protein, 24 aa, Homo sapiens
GAPPNSFEEFPFSALEGWTGATIT

SEQ ID NO: 5 - protein, 379 aa, Homo sapiens
NPNDKYEPFWEDEEKNESGLTEYRLVSINKSSPLQKQLPAFISEDASGYLTSSWLTLFVPSVYTGVFVVSLPLNIMAIVVFILKMKVKKPAVVYMLHLATADVLFVSVLPFKISYYFSGSDWQFGSELCRFVTAAFYCNMYASILLMTVISIDRFLAVVYPMQSLSWRTLGRASFTCLAIWALAIAGVVPLLLKEQTIQVPGLNITTCHDVLNETLLEGYYAYYFSAFSAVFFFVPLIISTVCYVSIIRCLSSSAVANRSKKSRALFLSAAVFCIFIICFGPTNVLLIAHYSFLSHTSTTEAAYFAYLLCVCVSSISCCIDPLIYYYASSECQRYVYSILCCKESSDPSSYNSSGQLMASKMDTCSSNLNNSIYKKLLT

SEQ ID NO: 6 - protein, 54 aa, Homo sapiens
NPNDKYEPFWEDEEKNESGLTEYRLVSINKSSPLQKQLPAFISEDASGYLTSSW

SEQ ID NO: 7 - protein, 20 aa, Homo sapiens
NPNDKYEPFWEDEEKNESGL

SEQ ID NO: 8 - protein, 13 aa, Homo sapiens
GAPPNSFEEFPFS

SEQ ID NO: 9 - protein, 15 aa, Homo sapiens
FPFSALEGWTGATIT

SEQ ID NO: 10 - protein, 9 aa, Homo sapiens
FPFSALEGW

SEQ ID NO: 11 - protein, 14 aa, Homo sapiens
GAPPNSFEEFPFSA

SEQ ID NO: 12 - protein, 15 aa, Homo sapiens
GAPPNSFEEFPFSAL

SEQ ID NO: 13 - protein, 16 aa, Homo sapiens
GAPPNSFEEFPFSALE

SEQ ID NO: 14 - protein, 17 aa, Homo sapiens
GAPPNSFEEFPFSALEG

SEQ ID NO: 15 - protein, 18 aa, Homo sapiens
GAPPNSFEEFPFSALEGW

SEQ ID NO: 16 - protein, 19 aa, Homo sapiens
GAPPNSFEEFPFSALEGWT

SEQ ID NO: 17 - protein, 20 aa, Homo sapiens
GAPPNSFEEFPFSALEGWTG

SEQ ID NO: 18 - protein, 21 aa, Homo sapiens
GAPPNSFEEFPFSALEGWTGA

SEQ ID NO: 19 - protein, 22 aa, Homo sapiens
GAPPNSFEEFPFSALEGWTGAT

SEQ ID NO: 20 - protein, 23 aa, Homo sapiens
GAPPNSFEEFPFSALEGWTGATI

SEQ ID NO: 21 - protein, 10 aa, Homo sapiens
FPFSALEGWT

SEQ ID NO: 22 - protein, 11 aa, Homo sapiens
FPFSALEGWTG

SEQ ID NO: 23 - protein, 12 aa, Homo sapiens
FPFSALEGWTGA

SEQ ID NO: 24 - protein, 13 aa, Homo sapiens
FPFSALEGWTGAT

SEQ ID NO: 25 - protein, 14 aa, Homo sapiens
FPFSALEGWTGATI

SEQ ID NO: 26 - protein, 8 aa, Homo sapiens
FPFSALEG

SEQ ID NO: 27 - protein, 7 aa, Homo sapiens
FPFSALE

SEQ ID NO: 28 - protein, 6 aa, Homo sapiens
FPFSAL

SEQ ID NO: 29 - protein, 7 aa, Homo sapiens
EFPFSAL

SEQ ID NO: 30 - protein, 8 aa, Homo sapiens
EEFPFSAL

SEQ ID NO: 31 - protein, 4 aa, Homo sapiens
NPND

SEQ ID NO: 32 - protein, 5 aa, Homo sapiens
NPNDK

SEQ ID NO: 33 - protein, 6 aa, Homo sapiens
NPNDKY

SEQ ID NO: 34 - protein, 7 aa, Homo sapiens
NPNDKYE

SEQ ID NO: 35 - protein, 8 aa, Homo sapiens
NPNDKYEP

SEQ ID NO: 36 - protein, 9 aa, Homo sapiens
NPNDKYEPF

SEQ ID NO: 37 - protein, 10 aa, Homo sapiens
NPNDKYEPFW

SEQ ID NO: 38 - protein, 11 aa, Homo sapiens
NPNDKYEPFWE

SEQ ID NO: 39 - protein, 12 aa, Homo sapiens
NPNDKYEPFWED

SEQ ID NO: 40 - protein, 13 aa, Homo sapiens
NPNDKYEPFWEDE

SEQ ID NO: 41 - protein, 14 aa, Homo sapiens
NPNDKYEPFWEDEE

SEQ ID NO: 42 - protein, 15 aa, Homo sapiens
NPNDKYEPFWEDEEK

SEQ ID NO: 43 - protein, 16 aa, Homo sapiens
NPNDKYEPFWEDEEKN

SEQ ID NO: 44 - protein, 17 aa, Homo sapiens
NPNDKYEPFWEDEEKNE

SEQ ID NO: 45 - protein, 18 aa, Homo sapiens
NPNDKYEPFWEDEEKNES

SEQ ID NO: 46 - protein, 19 aa, Homo sapiens
NPNDKYEPFWEDEEKNESG

SEQ ID NO: 47 - protein, 19 aa, Homo sapiens
PNDKYEPFWEDEEKNESGL

SEQ ID NO: 48 - protein, 15 aa, Homo sapiens
YEPFWEDEEKNESGL

SEQ ID NO: 49 - protein, 20 aa, synthetic construct
QPNDKYEPFWEDEEKNESGL

SEQ ID NO: 50 - protein, 20 aa, synthetic construct
APNDKYEPFWEDEEKNESGL

SEQ ID NO: 51 - protein, 18 aa, Homo sapiens
NDKYEPFWEDEEKNESGL

SEQ ID NO: 52 - protein, 20 aa, synthetic construct
DPNDKYEPFWEDEEKNESGL

SEQ ID NO: 53 - protein, 7 aa, Homo sapiens
PNDKYEP

SEQ ID NO: 54 - protein, 6 aa, Homo sapiens
SALEGW

SEQ ID NO: 55 - protein, 7 aa, Homo sapiens
WTGATIT

SEQ ID NO: 56 - protein, 20 aa, Homo sapiens
NPNDKYEPFWEDEEKNESGL

SEQ ID NO: 57 - protein, 17 aa, Homo sapiens
DKYEPFWEDEEKNESGL

SEQ ID NO: 58 - protein, 16 aa, Homo sapiens
KYEPFWEDEEKNESGL

SEQ ID NO: 59 - protein, 14 aa, Homo sapiens
EPFWEDEEKNESGL

SEQ ID NO: 60 - protein, 13 aa, Homo sapiens
PFWEDEEKNESGL

SEQ ID NO: 61 - protein, 34 aa, synthetic construct
NPNDKYEPFGGGGGGGGGGFPFSALEGWTGATIT